European Patent Specification EP 3 718 572 B1, published July 31, 2024. Title: Nucleic Acid,Composition and Conjugate Containing Nucleic Acid,Preparation Method and Use. Applicant: SU ZHOU RIBO LIFE SCIENCE CO.,LTD. The sequence listing filed with the application follows.

SEQUENCE LISTING (53 sequences)

SEQ ID NO: 1 - RNA, 19 nt, Artificial Sequence
  misc_feature (19)..(19): n is A
ugcuaugccucaucuucun

SEQ ID NO: 2 - RNA, 19 nt, Artificial Sequence
  misc_feature (1)..(1): n is U
nagaagaugaggcauagca

SEQ ID NO: 3 - RNA, 19 nt, Artificial Sequence
  misc_feature (19)..(19): n is selected from A,U,G and C
ugcuaugccucaucuucun

SEQ ID NO: 4 - RNA, 19 nt, Artificial Sequence
  misc_feature (1)..(1): n is selected from A,U,G and C
nagaagaugaggcauagca

SEQ ID NO: 5 - RNA, 21 nt, Artificial Sequence
  misc_feature (1)..(1): n is selected from A,U,G and C
nagaagaugaggcauagcagc

SEQ ID NO: 6 - RNA, 21 nt, Artificial Sequence
  misc_feature (1)..(1): n is selected from A,U,G and C
nagaagaugaggcauagcauu

SEQ ID NO: 7 - RNA, 21 nt, Artificial Sequence
  misc_feature (1)..(1): n is selected from A,U,G and C
nagaagaugaggcauagcagc

SEQ ID NO: 8 - RNA, 21 nt, Artificial Sequence
  misc_feature (1)..(1): n is selected from A,U,G and C
nagaagaugaggcauagcauu

SEQ ID NO: 9 - RNA, 19 nt, Artificial Sequence
ugcuaugccucaucuucua

SEQ ID NO: 10 - RNA, 21 nt, Artificial Sequence
uagaagaugaggcauagcagc

SEQ ID NO: 11 - RNA, 21 nt, Artificial Sequence
uagaagaugaggcauagcauu

SEQ ID NO: 12 - RNA, 19 nt, Artificial Sequence
ugcuaugccucaucuucua

SEQ ID NO: 13 - RNA, 21 nt, Artificial Sequence
uagaagaugaggcauagcagc

SEQ ID NO: 14 - RNA, 21 nt, Artificial Sequence
uagaagaugaggcauagcauu

SEQ ID NO: 15 - RNA, 19 nt, Artificial Sequence
ugcuaugccucaucuucua

SEQ ID NO: 16 - RNA, 21 nt, Artificial Sequence
uagaagaugaggcauagcagc

SEQ ID NO: 17 - RNA, 21 nt, Artificial Sequence
uagaagaugaggcauagcauu

SEQ ID NO: 18 - RNA, 19 nt, Artificial Sequence
ugcuaugccucaucuucua

SEQ ID NO: 19 - RNA, 21 nt, Artificial Sequence
uagaagaugaggcauagcagc

SEQ ID NO: 20 - RNA, 21 nt, Artificial Sequence
uagaagaugaggcauagcauu

SEQ ID NO: 21 - RNA, 21 nt, Artificial Sequence
uagaagaugaggcauagcagc

SEQ ID NO: 22 - RNA, 21 nt, Artificial Sequence
uagaagaugaggcauagcauu

SEQ ID NO: 23 - RNA, 21 nt, Artificial Sequence
uagaagaugaggcauagcagc

SEQ ID NO: 24 - RNA, 21 nt, Artificial Sequence
uagaagaugaggcauagcauu

SEQ ID NO: 25 - RNA, 21 nt, Artificial Sequence
uagaagaugaggcauagcagc

SEQ ID NO: 26 - RNA, 21 nt, Artificial Sequence
uagaagaugaggcauagcauu

SEQ ID NO: 27 - RNA, 21 nt, Artificial Sequence
uagaagaugaggcauagcagc

SEQ ID NO: 28 - RNA, 21 nt, Artificial Sequence
uagaagaugaggcauagcauu

SEQ ID NO: 29 - RNA, 21 nt, Artificial Sequence
uagaagaugaggcauagcagc

SEQ ID NO: 30 - RNA, 21 nt, Artificial Sequence
uagaagaugaggcauagcauu

SEQ ID NO: 31 - RNA, 21 nt, Artificial Sequence
uagaagaugaggcauagcagc

SEQ ID NO: 32 - RNA, 21 nt, Artificial Sequence
uagaagaugaggcauagcauu

SEQ ID NO: 33 - RNA, 21 nt, Artificial Sequence
uagaagaugaggcauagcagc

SEQ ID NO: 34 - RNA, 21 nt, Artificial Sequence
gcugcuaugccucaucuucua

SEQ ID NO: 35 - RNA, 23 nt, Artificial Sequence
uagaagaugaggcauagcagcgc

SEQ ID NO: 36 - RNA, 19 nt, Artificial Sequence
ugcuaugccucaucuucua

SEQ ID NO: 37 - RNA, 21 nt, Artificial Sequence
uagaagaugaggcauagcagc

SEQ ID NO: 38 - RNA, 19 nt, Artificial Sequence
ugcuaugccucaucuucua

SEQ ID NO: 39 - RNA, 21 nt, Artificial Sequence
uagaagaugaggcauagcauu

SEQ ID NO: 40 - RNA, 21 nt, Artificial Sequence
uagaagaugaggcauagcagc

SEQ ID NO: 41 - RNA, 21 nt, Artificial Sequence
uagaagaugaggcauagcagc

SEQ ID NO: 42 - RNA, 19 nt, Artificial Sequence
uucuccgaacgugucacgu

SEQ ID NO: 43 - RNA, 21 nt, Artificial Sequence
acgugacacguucggagaauu

SEQ ID NO: 44 - RNA, 19 nt, Artificial Sequence
gcugcuaugccucaucuua

SEQ ID NO: 45 - RNA, 21 nt, Artificial Sequence
uaagaugaggcauagcagcag

SEQ ID NO: 46 - RNA, 19 nt, Artificial Sequence
ccuugaggcauacuucaaa

SEQ ID NO: 47 - RNA, 21 nt, Artificial Sequence
uuugaaguaugccucaagguu

SEQ ID NO: 48 - DNA, 20 bp, Artificial Sequence
ccgtctgtgccttctcatct

SEQ ID NO: 49 - DNA, 20 bp, Artificial Sequence
taatctcctcccccaactcc

SEQ ID NO: 50 - DNA, 24 bp, Artificial Sequence
aactttggcattgtggaagggctc

SEQ ID NO: 51 - DNA, 24 bp, Artificial Sequence
tggaagagtgggagttgctgttga

SEQ ID NO: 52 - DNA, 21 bp, Artificial Sequence
cgtttctcctggctcagttta

SEQ ID NO: 53 - DNA, 21 bp, Artificial Sequence
cagcggtaaaaagggactcaa